European Patent Specification EP 4 005 584 B1, published October 11, 2023. Title: Use of amino acid sequences from Mycobacterium tuberculosis or corresponding nucleic acids thereof for diagnosis and prevention of tubercular infection, diagnostic kit and vaccine therefrom. Applicant: Mariani, Francesca Amicosante, Massimo Colizzi, Vittorio Saltini, Cesare. The sequence listing filed with the application follows.

SEQUENCE LISTING (87 sequences)

SEQ ID NO: 1 - protein, 20 aa, Mycobacterium tuberculosis
EMWDIRNRGVIPAGALPRVR

SEQ ID NO: 2 - protein, 30 aa, Mycobacterium tuberculosis
AKFRSVRVVVITGSVTAAPVRVSETLRRLI

SEQ ID NO: 3 - protein, 13 aa, Mycobacterium tuberculosis
ESVRLAFVAALQH

SEQ ID NO: 4 - protein, 14 aa, Mycobacterium tuberculosis
GLLITIRSPRSGIA

SEQ ID NO: 5 - protein, 13 aa, Mycobacterium tuberculosis
AQLLWQLPLLSIG

SEQ ID NO: 6 - protein, 27 aa, Mycobacterium tuberculosis
ADLVRELVTILPIVLVIAAVAAYLLSR

SEQ ID NO: 7 - protein, 20 aa, Mycobacterium tuberculosis
AAYLLSRAALRPVDRIRAAA

SEQ ID NO: 8 - protein, 20 aa, Mycobacterium tuberculosis
TTLNTMLTRLQRALAHEQQF

SEQ ID NO: 9 - protein, 21 aa, Mycobacterium tuberculosis
DLFVSIDPDHLRRILTAVLDN

SEQ ID NO: 10 - protein, 17 aa, Mycobacterium tuberculosis
SGLGLAIVAALTTTHGG

SEQ ID NO: 11 - protein, 19 aa, Mycobacterium tuberculosis
GRLPRKGPWQQKVIKELPQ

SEQ ID NO: 12 - protein, 20 aa, Mycobacterium tuberculosis
GKIVVLMGAVGTMKPETQAA

SEQ ID NO: 13 - protein, 14 aa, Mycobacterium tuberculosis
GEIIFISGRLNGAA

SEQ ID NO: 14 - protein, 13 aa, Mycobacterium tuberculosis
ARVRSMSPLEIAD

SEQ ID NO: 15 - protein, 15 aa, Mycobacterium tuberculosis
EQILFRRLAPFVGGF

SEQ ID NO: 16 - protein, 14 aa, Mycobacterium tuberculosis
AALVRALTACGCSS

SEQ ID NO: 17 - protein, 21 aa, Mycobacterium tuberculosis
DKWTLCQILYWRGVGTCISGD

SEQ ID NO: 18 - protein, 17 aa, Mycobacterium tuberculosis
TKVLGLYTQAQVLAYCG

SEQ ID NO: 19 - protein, 18 aa, Mycobacterium tuberculosis
DQVTMHQVLMAQLALAGG

SEQ ID NO: 20 - protein, 22 aa, Mycobacterium tuberculosis
EGVRLLGAAAALRQQTRQVRFK

SEQ ID NO: 21 - protein, 13 aa, Mycobacterium tuberculosis
ELMARAAVLGSAH

SEQ ID NO: 22 - protein, 13 aa, Mycobacterium tuberculosis
AVIVRSELLTQYL

SEQ ID NO: 23 - protein, 20 aa, Mycobacterium tuberculosis
GTLRHLDPPVRRSGGREQHL

SEQ ID NO: 24 - protein, 13 aa, Mycobacterium tuberculosis
TAWITAVVPGLMV

SEQ ID NO: 25 - protein, 13 aa, Mycobacterium tuberculosis
APMVFSATKGMTA

SEQ ID NO: 26 - protein, 14 aa, Mycobacterium tuberculosis
TCAMRRLAHRFSGG

SEQ ID NO: 27 - protein, 13 aa, Mycobacterium tuberculosis
SVVRRKQTLLSAQ

SEQ ID NO: 28 - protein, 13 aa, Mycobacterium tuberculosis
GVVHRNPAVTVAE

SEQ ID NO: 29 - protein, 22 aa, Mycobacterium tuberculosis
PGVVATHAVRTLGTTGSRAIGL

SEQ ID NO: 30 - protein, 25 aa, Mycobacterium tuberculosis
PQWRRARVRLCGRWWRRSNTTRGAS

SEQ ID NO: 31 - protein, 18 aa, Mycobacterium tuberculosis
ARLMVGAVRRHRPGSLQR

SEQ ID NO: 32 - protein, 12 aa, Mycobacterium tuberculosis
AAMRNMKSTSHE

SEQ ID NO: 33 - protein, 14 aa, Mycobacterium tuberculosis
QTIVMLWTAAVGCA

SEQ ID NO: 34 - protein, 19 aa, Mycobacterium tuberculosis
LCMLMLGLLMLIFSEHRSS

SEQ ID NO: 35 - protein, 20 aa, Mycobacterium tuberculosis
SALVLVGLGLCGSGVALCLT

SEQ ID NO: 36 - protein, 16 aa, Mycobacterium tuberculosis
SELVRFELLAGVRESE

SEQ ID NO: 37 - protein, 14 aa, Mycobacterium tuberculosis
VDYLIAATAIVVDA

SEQ ID NO: 38 - protein, 15 aa, Mycobacterium tuberculosis
QGIEYYKSSVLPQIE

SEQ ID NO: 39 - protein, 16 aa, Mycobacterium tuberculosis
EGWIVYARSTTIQAQS

SEQ ID NO: 40 - protein, 10 aa, Mycobacterium tuberculosis
TRRMYSNYGF

SEQ ID NO: 41 - protein, 23 aa, Mycobacterium tuberculosis
FGYRVQESAFEAMLTKGQLAKLV

SEQ ID NO: 42 - protein, 26 aa, Mycobacterium tuberculosis
DNIRIYKIRGVAAVTFYGRGRLVSAE

SEQ ID NO: 43 - protein, 23 aa, Mycobacterium tuberculosis
RSYILRAGISSLFRYIEGVHGER

SEQ ID NO: 44 - protein, 20 aa, Mycobacterium tuberculosis
SAMRPQDRLLVGNWVDDSLL

SEQ ID NO: 45 - protein, 13 aa, Mycobacterium tuberculosis
LYLVGLEPYVQFE

SEQ ID NO: 46 - protein, 13 aa, Mycobacterium tuberculosis
AGFRILEARRFPI

SEQ ID NO: 47 - protein, 19 aa, Mycobacterium tuberculosis
IRYRARYVNGQLNMCLARI

SEQ ID NO: 48 - protein, 16 aa, Mycobacterium tuberculosis
ALLVAYLPARSREEMF

SEQ ID NO: 49 - protein, 13 aa, Mycobacterium tuberculosis
NRLRLAATHAVRT

SEQ ID NO: 50 - protein, 21 aa, Mycobacterium tuberculosis
APLQRRFRDAFTATAHFQVNE

SEQ ID NO: 51 - protein, 18 aa, Mycobacterium tuberculosis
SRELPGRVLLDQPADVSM

SEQ ID NO: 52 - protein, 18 aa, Mycobacterium tuberculosis
EPVVTVDVTAMSAVLEID

SEQ ID NO: 53 - protein, 23 aa, Mycobacterium tuberculosis
AVIQVSDRAVRGWRTGDIRPERY

SEQ ID NO: 54 - protein, 17 aa, Mycobacterium tuberculosis
PDLRGALLLAVTLGLVT

SEQ ID NO: 55 - protein, 16 aa, Mycobacterium tuberculosis
PDWGWLSVATVGSFLA

SEQ ID NO: 56 - protein, 21 aa, Mycobacterium tuberculosis
GAVLGVAVMVILIGKPEHGTA

SEQ ID NO: 57 - protein, 15 aa, Mycobacterium tuberculosis
AAICFIAVAVAAAVL

SEQ ID NO: 58 - protein, 15 aa, Mycobacterium tuberculosis
TKLVRLTKAQFDEIA

SEQ ID NO: 59 - protein, 14 aa, Mycobacterium tuberculosis
ADLVLAGPAASREH

SEQ ID NO: 60 - protein, 16 aa, Mycobacterium tuberculosis
YAYEYFIRHNPLSDYA

SEQ ID NO: 61 - protein, 18 aa, Mycobacterium tuberculosis
FPVRGLVRGRRTLTLLEA

SEQ ID NO: 62 - protein, 16 aa, Mycobacterium tuberculosis
EVLRILRRRSLAALRA

SEQ ID NO: 63 - protein, 18 aa, Mycobacterium tuberculosis
RVILHSPYGLRVHGPLAL

SEQ ID NO: 64 - protein, 15 aa, Mycobacterium tuberculosis
AAWVINGLANAYNDT

SEQ ID NO: 65 - protein, 27 aa, Mycobacterium tuberculosis
DQYRARNVAVMNAYVSWTRSALSDLPR

SEQ ID NO: 66 - protein, 25 aa, Mycobacterium tuberculosis
SDLLADAVERYLQWLSKSSSQLKHA

SEQ ID NO: 67 - protein, 13 aa, Mycobacterium tuberculosis
GPVVVHPSWWSAA

SEQ ID NO: 68 - protein, 16 aa, Mycobacterium tuberculosis
ITAVVLIDVPSTVAGA

SEQ ID NO: 69 - protein, 14 aa, Mycobacterium tuberculosis
AAVVRHGATTLQRP

SEQ ID NO: 70 - protein, 18 aa, Mycobacterium tuberculosis
RPVRRVLLFVVPSSGPAP

SEQ ID NO: 71 - protein, 24 aa, Mycobacterium tuberculosis
GSVRQLPSVLKPPLITLRTLTLSG

SEQ ID NO: 72 - protein, 18 aa, Mycobacterium tuberculosis
GAVLRLVVRFAEPLPPSP

SEQ ID NO: 73 - protein, 19 aa, Mycobacterium tuberculosis
AGYLLTYTIANNGKEFAEL

SEQ ID NO: 74 - protein, 18 aa, Mycobacterium tuberculosis
AAVRKRMVIGLSTGSDDD

SEQ ID NO: 75 - protein, 20 aa, Mycobacterium tuberculosis
ALLLRDVLQWKSAEVADAIG

SEQ ID NO: 76 - protein, 25 aa, Mycobacterium tuberculosis
NSLLQRARSQLQTVRPSAADRLSAA

SEQ ID NO: 77 - protein, 20 aa, Mycobacterium tuberculosis
MSWVMVSPELVVAAAADLAG

SEQ ID NO: 78 - protein, 17 aa, Mycobacterium tuberculosis
AAFYAQFVQALTSGGAY

SEQ ID NO: 79 - protein, 14 aa, Mycobacterium tuberculosis
ALLVRMPTSLPAVA

SEQ ID NO: 80 - protein, 27 aa, Mycobacterium tuberculosis
SRLRTHVRPDAPLVPLALRVDGLRSRW

SEQ ID NO: 81 - protein, 14 aa, Mycobacterium tuberculosis
AAVLTMLGVAGYGW

SEQ ID NO: 82 - protein, 21 aa, Mycobacterium tuberculosis
GLFMIFLDALIVNVALPDIQR

SEQ ID NO: 83 - protein, 25 aa, Mycobacterium tuberculosis
SWVVASYSLGMAVFIMSAGTLADLL

SEQ ID NO: 84 - protein, 25 aa, Mycobacterium tuberculosis
QQWNFAGIEAAASAIQGNVTSIHSL

SEQ ID NO: 85 - protein, 13 aa, Mycobacterium tuberculosis
LAWITAVVPGLMV

SEQ ID NO: 86 - protein, 12 aa, Mycobacterium tuberculosis
GEIIFISGRLNG

SEQ ID NO: 87 - protein, 14 aa, Mycobacterium tuberculosis
SALLRRLSTCPPES